European Patent Specification EP 3 344 655 B1, published July 26, 2023. Title: Anti-CD40 Antibodies. Applicant: Brodeur, Scott. The sequence listing filed with the application follows.

SEQUENCE LISTING (78 sequences)

SEQ ID NO: 1 - protein, 118 aa, Artificial Sequence
  CD40 Murine Lead VH Sequence of 2H11
EVQLQQSGAELVRPGASVKLSCTASGFNIKDYYVHWVKQRPEKGLEWIGRIDPEDGDSKYAPKFQGKATMTADTSSNTAYLHLSSLTSEDTAVYYCTTSYYVGTYGYWGQGTTLTVSS

SEQ ID NO: 2 - protein, 118 aa, Artificial Sequence
  CD40 Murine Lead VH Sequence of 10F2
EVQLQQSGAELVRPGASVKLSCTASGFNIKDYYIHWVKQRPEKGLEWIGRIDPEDGDTKYDPKFQGKATMTADTSSNTAYLHLSSLTSEDTAVYYCTTSYYVGTYGYWGQGTTLTVSS

SEQ ID NO: 3 - protein, 118 aa, Artificial Sequence
  CD40 Murine Lead VH Sequence of 19B10
EVQLQQSGAELVRPGASVQLSCTASGFNIKDYYVHWVKQRPEKGLEWIGRIDPEDGDTKFAPKFQGKATMTADTSSNTVYLHLSSLTSEDTAVYYCTTSYYVGTYGYWGQGTTLTVSS

SEQ ID NO: 4 - protein, 119 aa, Artificial Sequence
  CD40 Murine Lead VH Sequence of 20E2
EVQLVESGGGLVKPGGSRKLSCAASGFTFSDYGMHWVRQAPEKGLEWVAYISSGNRIIYYADTVKGRFTISRDNAKNTLFLQMTSLRSEDTALYYCARQDGYRYAMDYWGQGTSVTVSS

SEQ ID NO: 5 - protein, 106 aa, Artificial Sequence
  CD40 Murine Lead VK Sequence of 2H11
QIVLTQSPAIMSASPGEKVTITCSASSSVSYMLWFQQKPGTSPKLWIYSTSNLASGVPARFGGSGSGTSYSLTISRMEAEDAATYYCQQRTFYPYTFGGGTKLEIK

SEQ ID NO: 6 - protein, 106 aa, Artificial Sequence
  CD40 Murine Lead VK Sequence of 10F2
QIVLTQSPTIMSASPGEKVIITCSATSSVSYILWFQQKPGTSPKLWIYSTSNLASGVPARFSGSGSGASYSLTISRMEAEDAATYYCQQRTFYPYTFGGGTKLEIK

SEQ ID NO: 7 - protein, 106 aa, Artificial Sequence
  CD40 Murine Lead VK Sequence of 19B10
QIVLTQSPAIMSASPGEKVTITCSASSSVSYMLWFQQKPGTSPKLWIYSTSNLASGVPARFSGSGSGTSYSLTISRMEAEDAATYYCQQRTFYPYTFGGGTKLEIK

SEQ ID NO: 8 - protein, 113 aa, Artificial Sequence
  CD40 Murine Lead VK Sequence of 20E2
DIVMTQSPSSLTVTAGEKVTMSCKSSQSLLNSGNQKNYLTWHQQKPGQPPKLLIYWTSTRESGVPDRFTGSGSGTDFTLTISNLQAEDLAVYYCQNDYTYPLTFGAGTKLELK

SEQ ID NO: 9 - protein, 10 aa, Artificial Sequence
  CDR1 Heavy Chain of 2H11 and 19B10
GFNIKDYYVH

SEQ ID NO: 10 - protein, 10 aa, Artificial Sequence
  CDR1 Heavy Chain of 10F2
GFNIKDYYIH

SEQ ID NO: 11 - protein, 10 aa, Artificial Sequence
  CDR1 Heavy Chain of 20E2
GFTFSDYGMH

SEQ ID NO: 12 - protein, 17 aa, Artificial Sequence
  CDR2 Heavy Chain of 2H11
RIDPEDGDSKYAPKFQG

SEQ ID NO: 13 - protein, 17 aa, Artificial Sequence
  CDR2 Heavy Chain of 10F2
RIDPEDGDTKYDPKFQG

SEQ ID NO: 14 - protein, 17 aa, Artificial Sequence
  CDR2 Heavy Chain of 19B10
RIDPEDGDTKFAPKFQG

SEQ ID NO: 15 - protein, 17 aa, Artificial Sequence
  CDR2 Heavy Chain of 20E2
YISSGNRIIYYADTVKG

SEQ ID NO: 16 - protein, 9 aa, Artificial Sequence
  CDR3 Heavy Chain of 2H11, 10F2 and 19B10
SYYVGTYGY

SEQ ID NO: 17 - protein, 10 aa, Artificial Sequence
  CDR3 Heavy Chain of 20E2
QDGYRYAMDY

SEQ ID NO: 18 - protein, 10 aa, Artificial Sequence
  CDR1 Light Chain of 2H11
SASSSVSYML

SEQ ID NO: 19 - protein, 10 aa, Artificial Sequence
  CDR1 Light Chain of 10F2
SATSSVSYIL

SEQ ID NO: 20 - protein, 10 aa, Artificial Sequence
  CDR1 Light Chain of 19B10
SASSSVSYML

SEQ ID NO: 21 - protein, 17 aa, Artificial Sequence
  CDR1 Light Chain of 20E2
KSSQSLLNSGNQKNYLT

SEQ ID NO: 22 - protein, 7 aa, Artificial Sequence
  CDR2 Light Chain of 2H11, 10F2 and 19B10
STSNLAS

SEQ ID NO: 23 - protein, 7 aa, Artificial Sequence
  CDR2 Light Chain of 20E2
WTSTRES

SEQ ID NO: 24 - protein, 9 aa, Artificial Sequence
  CDR3 Light Chain of 2H11, 10F2, and 19B10
QQRTFYPYT

SEQ ID NO: 25 - protein, 9 aa, Artificial Sequence
  CDR3 Light Chain of 20E2
QNDYTYPLT

SEQ ID NO: 26 - protein, 220 aa, Artificial Sequence
  Light Chain of Antibody A
DIVMTQSPDSLAVSLGERATMSCKSSQSLLNSGNQKNYLTWHQQKPGQPPKLLIYWTSTRESGVPDRFSGSGSGTDFTLTISSLQAEDVAVYYCQNDYTYPLTFGGGTKVEIKRTVAAPSVFIFPPSDEQLKSGTASVVCLLNNFYPREAKVQWKVDNALQSGNSQESVTEQDSKDSTYSLSSTLTLSKADYEKHKVYACEVTHQGLSSPVTKSFNRGEC

SEQ ID NO: 27 - protein, 449 aa, Artificial Sequence
  Heavy Chain IgG1K0 of Antibody A
EVQLVESGGGLVKPGGSLRLSCAASGFTFSDYGMHWVRQAPGKGLEWVAYISSGNRIIYYADTVKGRFTISRDNAKNSLYLQMNSLRAEDTALYYCARQDGYRYAMDYWAQGTLVTVSSASTKGPSVFPLAPSSKSTSGGTAALGCLVKDYFPEPVTVSWNSGALTSGVHTFPAVLQSSGLYSLSSVVTVPSSSLGTQTYICNVNHKPSNTKVDKRVEPKSCDKTHTCPPCPAPEAAGGPSVFLFPPKPKDTLMISRTPEVTCVVVDVSHEDPEVKFNWYVDGVEVHNAKTKPREEQYNSTYRVVSVLTVLHQDWLNGKEYKCKVSNKALPAPIEKTISKAKGQPREPQVYTLPPSREEMTKNQVSLTCLVKGFYPSDIAVEWESNGQPENNYKTTPPVLDSDGSFFLYSKLTVDKSRWQQGNVFSCSVMHEALHNHYTQKSLSLSPGK

SEQ ID NO: 28 - protein, 449 aa, Artificial Sequence
  Heavy Chain IgG1 of Antibody A
EVQLVESGGGLVKPGGSLRLSCAASGFTFSDYGMHWVRQAPGKGLEWVAYISSGNRIIYYADTVKGRFTISRDNAKNSLYLQMNSLRAEDTALYYCARQDGYRYAMDYWAQGTLVTVSSASTKGPSVFPLAPSSKSTSGGTAALGCLVKDYFPEPVTVSWNSGALTSGVHTFPAVLQSSGLYSLSSVVTVPSSSLGTQTYICNVNHKPSNTKVDKRVEPKSCDKTHTCPPCPAPELLGGPSVFLFPPKPKDTLMISRTPEVTCVVVDVSHEDPEVKFNWYVDGVEVHNAKTKPREEQYNSTYRVVSVLTVLHQDWLNGKEYKCKVSNKALPAPIEKTISKAKGQPREPQVYTLPPSREEMTKNQVSLTCLVKGFYPSDIAVEWESNGQPENNYKTTPPVLDSDGSFFLYSKLTVDKSRWQQGNVFSCSVMHEALHNHYTQKSLSLSPGK

SEQ ID NO: 29 - protein, 446 aa, Artificial Sequence
  Heavy Chain IgG4DM of Antibody A
EVQLVESGGGLVKPGGSLRLSCAASGFTFSDYGMHWVRQAPGKGLEWVAYISSGNRIIYYADTVKGRFTISRDNAKNSLYLQMNSLRAEDTALYYCARQDGYRYAMDYWAQGTLVTVSSASTKGPSVFPLAPCSRSTSESTAALGCLVKDYFPEPVTVSWNSGALTSGVHTFPAVLQSSGLYSLSSVVTVPSSSLGTKTYTCNVDHKPSNTKVDKRVESKYGPPCPPCPAPEFEGGPSVFLFPPKPKDTLMISRTPEVTCVVVDVSQEDPEVQFNWYVDGVEVHNAKTKPREEQFNSTYRVVSVLTVLHQDWLNGKEYKCKVSNKGLPSSIEKTISKAKGQPREPQVYTLPPSQEEMTKNQVSLTCLVKGFYPSDIAVEWESNGQPENNYKTTPPVLDSDGSFFLYSRLTVDKSRWQEGNVFSCSVMHEALHNHYTQKSLSLSLGK

SEQ ID NO: 30 - protein, 449 aa, Artificial Sequence
  Heavy Chain IgG1K0b of Antibody A
EVQLVESGGGLVKPGGSLRLSCAASGFTFSDYGMHWVRQAPGKGLEWVAYISSGNRIIYYADTVKGRFTISRDNAKNSLYLQMNSLRAEDTALYYCARQDGYRYAMDYWAQGTLVTVSSASTKGPSVFPLAPSSKSTSGGTAALGCLVKDYFPEPVTVSWNSGALTSGVHTFPAVLQSSGLYSLSSVVTVPSSSLGTQTYICNVNHKPSNTKVDKRVEPKSCDKTHTCPPCPAPEAAGGPSVFLFPPKPKDTLMISRTPEVTCVVVDVSHEDPEVKFNWYVDGVEVHNAKTKPREEQYNSTYRVVSVLTVLHQDWLNGKEYKCKVSNKALPAPIEKTISKAKGQPREPQVYTLPPSRDELTKNQVSLTCLVKGFYPSDIAVEWESNGQPENNYKTTPPVLDSDGSFFLYSKLTVDKSRWQQGNVFSCSVMHEALHNHYTQKSLSLSPGK

SEQ ID NO: 31 - protein, 220 aa, Artificial Sequence
  Light Chain of Antibody B
DIVMTQSPDSLAVSLGEKVTINCKSSQSLLNSGNQKNYLTWHQQKPGQPPKLLIYWTSTRESGVPDRFSGSGSGTDFTLTISSLQAEDVAVYYCQNDYTYPLTFGGGTKVEIKRTVAAPSVFIFPPSDEQLKSGTASVVCLLNNFYPREAKVQWKVDNALQSGNSQESVTEQDSKDSTYSLSSTLTLSKADYEKHKVYACEVTHQGLSSPVTKSFNRGEC

SEQ ID NO: 32 - protein, 449 aa, Artificial Sequence
  Heavy Chain IgG1K0 of Antibody B
EVQLVESGGGLVKPGGSLRLSCAASGFTFSDYGMHWVRQAPGKGLEWVAYISSGNRIIYYADTVKGRFTISRDNAKNSLYLQMNSLRAEDTAVYYCARQDGYRYAMDYWGQGTLVTVSSASTKGPSVFPLAPSSKSTSGGTAALGCLVKDYFPEPVTVSWNSGALTSGVHTFPAVLQSSGLYSLSSVVTVPSSSLGTQTYICNVNHKPSNTKVDKRVEPKSCDKTHTCPPCPAPEAAGGPSVFLFPPKPKDTLMISRTPEVTCVVVDVSHEDPEVKFNWYVDGVEVHNAKTKPREEQYNSTYRVVSVLTVLHQDWLNGKEYKCKVSNKALPAPIEKTISKAKGQPREPQVYTLPPSREEMTKNQVSLTCLVKGFYPSDIAVEWESNGQPENNYKTTPPVLDSDGSFFLYSKLTVDKSRWQQGNVFSCSVMHEALHNHYTQKSLSLSPGK

SEQ ID NO: 33 - protein, 449 aa, Artificial Sequence
  Heavy Chain IgG1 of Antibody B
EVQLVESGGGLVKPGGSLRLSCAASGFTFSDYGMHWVRQAPGKGLEWVAYISSGNRIIYYADTVKGRFTISRDNAKNSLYLQMNSLRAEDTAVYYCARQDGYRYAMDYWGQGTLVTVSSASTKGPSVFPLAPSSKSTSGGTAALGCLVKDYFPEPVTVSWNSGALTSGVHTFPAVLQSSGLYSLSSVVTVPSSSLGTQTYICNVNHKPSNTKVDKRVEPKSCDKTHTCPPCPAPELLGGPSVFLFPPKPKDTLMISRTPEVTCVVVDVSHEDPEVKFNWYVDGVEVHNAKTKPREEQYNSTYRVVSVLTVLHQDWLNGKEYKCKVSNKALPAPIEKTISKAKGQPREPQVYTLPPSREEMTKNQVSLTCLVKGFYPSDIAVEWESNGQPENNYKTTPPVLDSDGSFFLYSKLTVDKSRWQQGNVFSCSVMHEALHNHYTQKSLSLSPGK

SEQ ID NO: 34 - protein, 446 aa, Artificial Sequence
  Heavy Chain IgG4DM of Antibody B
EVQLVESGGGLVKPGGSLRLSCAASGFTFSDYGMHWVRQAPGKGLEWVAYISSGNRIIYYADTVKGRFTISRDNAKNSLYLQMNSLRAEDTAVYYCARQDGYRYAMDYWGQGTLVTVSSASTKGPSVFPLAPCSRSTSESTAALGCLVKDYFPEPVTVSWNSGALTSGVHTFPAVLQSSGLYSLSSVVTVPSSSLGTKTYTCNVDHKPSNTKVDKRVESKYGPPCPPCPAPEFEGGPSVFLFPPKPKDTLMISRTPEVTCVVVDVSQEDPEVQFNWYVDGVEVHNAKTKPREEQFNSTYRVVSVLTVLHQDWLNGKEYKCKVSNKGLPSSIEKTISKAKGQPREPQVYTLPPSQEEMTKNQVSLTCLVKGFYPSDIAVEWESNGQPENNYKTTPPVLDSDGSFFLYSRLTVDKSRWQEGNVFSCSVMHEALHNHYTQKSLSLSLGK

SEQ ID NO: 35 - protein, 449 aa, Artificial Sequence
  Heavy Chain IgG1K0b of Antibody B
EVQLVESGGGLVKPGGSLRLSCAASGFTFSDYGMHWVRQAPGKGLEWVAYISSGNRIIYYADTVKGRFTISRDNAKNSLYLQMNSLRAEDTAVYYCARQDGYRYAMDYWGQGTLVTVSSASTKGPSVFPLAPSSKSTSGGTAALGCLVKDYFPEPVTVSWNSGALTSGVHTFPAVLQSSGLYSLSSVVTVPSSSLGTQTYICNVNHKPSNTKVDKRVEPKSCDKTHTCPPCPAPEAAGGPSVFLFPPKPKDTLMISRTPEVTCVVVDVSHEDPEVKFNWYVDGVEVHNAKTKPREEQYNSTYRVVSVLTVLHQDWLNGKEYKCKVSNKALPAPIEKTISKAKGQPREPQVYTLPPSRDELTKNQVSLTCLVKGFYPSDIAVEWESNGQPENNYKTTPPVLDSDGSFFLYSKLTVDKSRWQQGNVFSCSVMHEALHNHYTQKSLSLSPGK

SEQ ID NO: 36 - protein, 213 aa, Artificial Sequence
  Light Chain of Antibody C
DIQMTQSPSSLSASVGDRVTITCSASSSVSYMLWFQQKPGKAPKLLIYSTSNLASGVPSRFSGSGSGTDFTLTISSLQPEDFATYYCQQRTFYPYTFGGGTKVEIKRTVAAPSVFIFPPSDEQLKSGTASVVCLLNNFYPREAKVQWKVDNALQSGNSQESVTEQDSKDSTYSLSSTLTLSKADYEKHKVYACEVTHQGLSSPVTKSFNRGEC

SEQ ID NO: 37 - protein, 448 aa, Artificial Sequence
  Heavy Chain IgG1K0 of Antibody C
QVQLVQSGAEVKKPGASVKVSCTASGFNIKDYYVHWVKQAPGQGLEWMGRIDPEDGDSKYAPKFQGKATMTADTSTSTVYMELSSLRSEDTAVYYCTTSYYVGTYGYWGQGTLVTVSSASTKGPSVFPLAPSSKSTSGGTAALGCLVKDYFPEPVTVSWNSGALTSGVHTFPAVLQSSGLYSLSSVVTVPSSSLGTQTYICNVNHKPSNTKVDKRVEPKSCDKTHTCPPCPAPEAAGGPSVFLFPPKPKDTLMISRTPEVTCVVVDVSHEDPEVKFNWYVDGVEVHNAKTKPREEQYNSTYRVVSVLTVLHQDWLNGKEYKCKVSNKALPAPIEKTISKAKGQPREPQVYTLPPSREEMTKNQVSLTCLVKGFYPSDIAVEWESNGQPENNYKTTPPVLDSDGSFFLYSKLTVDKSRWQQGNVFSCSVMHEALHNHYTQKSLSLSPGK

SEQ ID NO: 38 - protein, 448 aa, Artificial Sequence
  Heavy Chain IgG1 of Antibody C
QVQLVQSGAEVKKPGASVKVSCTASGFNIKDYYVHWVKQAPGQGLEWMGRIDPEDGDSKYAPKFQGKATMTADTSTSTVYMELSSLRSEDTAVYYCTTSYYVGTYGYWGQGTLVTVSSASTKGPSVFPLAPSSKSTSGGTAALGCLVKDYFPEPVTVSWNSGALTSGVHTFPAVLQSSGLYSLSSVVTVPSSSLGTQTYICNVNHKPSNTKVDKRVEPKSCDKTHTCPPCPAPELLGGPSVFLFPPKPKDTLMISRTPEVTCVVVDVSHEDPEVKFNWYVDGVEVHNAKTKPREEQYNSTYRVVSVLTVLHQDWLNGKEYKCKVSNKALPAPIEKTISKAKGQPREPQVYTLPPSREEMTKNQVSLTCLVKGFYPSDIAVEWESNGQPENNYKTTPPVLDSDGSFFLYSKLTVDKSRWQQGNVFSCSVMHEALHNHYTQKSLSLSPGK

SEQ ID NO: 39 - protein, 445 aa, Artificial Sequence
  Heavy Chain IgG4DM of Antibody C
QVQLVQSGAEVKKPGASVKVSCTASGFNIKDYYVHWVKQAPGQGLEWMGRIDPEDGDSKYAPKFQGKATMTADTSTSTVYMELSSLRSEDTAVYYCTTSYYVGTYGYWGQGTLVTVSSASTKGPSVFPLAPCSRSTSESTAALGCLVKDYFPEPVTVSWNSGALTSGVHTFPAVLQSSGLYSLSSVVTVPSSSLGTKTYTCNVDHKPSNTKVDKRVESKYGPPCPPCPAPEFEGGPSVFLFPPKPKDTLMISRTPEVTCVVVDVSQEDPEVQFNWYVDGVEVHNAKTKPREEQFNSTYRVVSVLTVLHQDWLNGKEYKCKVSNKGLPSSIEKTISKAKGQPREPQVYTLPPSQEEMTKNQVSLTCLVKGFYPSDIAVEWESNGQPENNYKTTPPVLDSDGSFFLYSRLTVDKSRWQEGNVFSCSVMHEALHNHYTQKSLSLSLGK

SEQ ID NO: 40 - protein, 448 aa, Artificial Sequence
  Heavy Chain IgG1K0b of Antibody C
QVQLVQSGAEVKKPGASVKVSCTASGFNIKDYYVHWVKQAPGQGLEWMGRIDPEDGDSKYAPKFQGKATMTADTSTSTVYMELSSLRSEDTAVYYCTTSYYVGTYGYWGQGTLVTVSSASTKGPSVFPLAPSSKSTSGGTAALGCLVKDYFPEPVTVSWNSGALTSGVHTFPAVLQSSGLYSLSSVVTVPSSSLGTQTYICNVNHKPSNTKVDKRVEPKSCDKTHTCPPCPAPEAAGGPSVFLFPPKPKDTLMISRTPEVTCVVVDVSHEDPEVKFNWYVDGVEVHNAKTKPREEQYNSTYRVVSVLTVLHQDWLNGKEYKCKVSNKALPAPIEKTISKAKGQPREPQVYTLPPSRDELTKNQVSLTCLVKGFYPSDIAVEWESNGQPENNYKTTPPVLDSDGSFFLYSKLTVDKSRWQQGNVFSCSVMHEALHNHYTQKSLSLSPGK

SEQ ID NO: 41 - protein, 113 aa, Artificial Sequence
  Variable Light Chain
DIVMTQSPDSLAVSLGERVTMSCKSSQSLLNSGNQKNYLTWHQQKPGQPPKLLIYWTSTRESGVPDRFSGSGSGTDFTLTISSLQAEDVAVYYCQNDYTYPLTFGGGTKVEIK

SEQ ID NO: 42 - protein, 119 aa, Artificial Sequence
  Variable Heavy Chain
EVQLVKSGGGLVKPGGSLRLSCAASGFTFSDYGMHWVRQAPGKGLEWVAYISSGNRIIYYADTVKGRFTISRDNAKNSLYLQMNSLRAEDTALYYCARQDGYRYAMDYWGQGTLVTVSS

SEQ ID NO: 43 - protein, 113 aa, Artificial Sequence
  Variable Light Chain in Antibody A
DIVMTQSPDSLAVSLGERATMSCKSSQSLLNSGNQKNYLTWHQQKPGQPPKLLIYWTSTRESGVPDRFSGSGSGTDFTLTISSLQAEDVAVYYCQNDYTYPLTFGGGTKVEIK

SEQ ID NO: 44 - protein, 119 aa, Artificial Sequence
  Variable Heavy Chain Antibody A
EVQLVESGGGLVKPGGSLRLSCAASGFTFSDYGMHWVRQAPGKGLEWVAYISSGNRIIYYADTVKGRFTISRDNAKNSLYLQMNSLRAEDTALYYCARQDGYRYAMDYWAQGTLVTVSS

SEQ ID NO: 45 - protein, 113 aa, Artificial Sequence
  Variable Light Chain
DIVMTQSPDSLAVSLGEKVTMNCKSSQSLLNSGNQKNYLTWHQQKPGQPPKLLIYWTSTRESGVPDRFSGSGSGTDFTLTISSLQAEDVAVYYCQNDYTYPLTFGAGTKVEIK

SEQ ID NO: 46 - protein, 119 aa, Artificial Sequence
  Variable Heavy Chain
EVQLVESGGGLVKPGGSRRLSCAASGFTFSDYGMHWVRQAPGKGLEWVAYISSGNRIIYYADTVKGRFTISRDNAKNSLYLQMNSLRAEDTALYYCARQDGYRYAMDYWGQGTLVTVSS

SEQ ID NO: 47 - protein, 113 aa, Artificial Sequence
  Variable Light Chain
DIVMTQSPDSLAVSLGERVTMNCKSSQSLLNSGNQKNYLTWHQQKPGQPPKLLIYWTSTRESGVPDRFSGSGSGTDFTLTISSLQAEDVAVYYCQNDYTYPLTFGGGTKVEIK

SEQ ID NO: 48 - protein, 119 aa, Artificial Sequence
  Variable Heavy Chain
EVQLVESGGGLVKPGGSLRLSCAASGFTFSDYGMHWVRQAPGKGLEWVAYISSGNRIIYYADTVKGRFTISRDNAKNSLYLQMNSLRAEDTALYYCARQDGYRYAMDYWGQGTLVTVSS

SEQ ID NO: 49 - protein, 113 aa, Artificial Sequence
  Variable Light Chain
DIVMTQSPDSLAVSLGERVTMNCKSSQSLLNSGNQKNYLTWHQQKPGQPPKLLIYWTSTRESGVPDRFSGSGSGTDFTLTISSLQAEDVAVYYCQNDYTYPLTFGAGTKVEIK

SEQ ID NO: 50 - protein, 119 aa, Artificial Sequence
  Variable Light Chain
EVQLVESGGGLVKPGGSRRLSCAASGFTFSDYGMHWVRQAPGKGLEWVAYISSGNRIIYYADTVKGRFTISRDNAKNSLYLQMNSLRAEDTAVYYCARQDGYRYAMDYWGQGTLVTVSS

SEQ ID NO: 51 - protein, 113 aa, Artificial Sequence
  Variable Light Chain
DIVMTQSPDSLAVSLGEKVTMNCKSSQSLLNSGNQKNYLTWHQQKPGQPPKLLIYWTSTRESGVPDRFSGSGSGTDFTLTISSLQAEDLAVYYCQNDYTYPLTFGAGTKVEIK

SEQ ID NO: 52 - protein, 113 aa, Artificial Sequence
  Variable Light Chain in Antibody B
DIVMTQSPDSLAVSLGEKVTINCKSSQSLLNSGNQKNYLTWHQQKPGQPPKLLIYWTSTRESGVPDRFSGSGSGTDFTLTISSLQAEDVAVYYCQNDYTYPLTFGGGTKVEIK

SEQ ID NO: 53 - protein, 119 aa, Artificial Sequence
  Variable Heavy Chain
EVQLVESGGGLVKPGGSLRLSCAASGFTFSDYGMHWVRQAPGKGLEWVAYISSGNRIIYYADTVKGRFTISRDNAKNSLYLQMNSLRAEDTAVYYCARQDGYRYAMDYWGQGTLVTVSS

SEQ ID NO: 54 - protein, 106 aa, Artificial Sequence
  Variable Light Chain
QIQMTQSPSSLSASVGDRVTITCSASSSVSYMLWFQQKPGKAPKLWIYSTSNLASGVPARFSGSGSGTDFTLTISSLQPEDFATYYCQQRTFYPYTFGGGTKVEIK

SEQ ID NO: 55 - protein, 106 aa, Artificial Sequence
  Variable Light Chain
DIQMTQSPSSLSASVGDRVTITCSASSSVSYMLWFQQKPGKAPKLLIYSTSNLASGVPARFSGSGSGTDFTLTISSLQPEDFATYYCQQRTFYPYTFGGGTKVEIK

SEQ ID NO: 56 - protein, 106 aa, Artificial Sequence
  Variable Light Chain
DIQMTQSPSSLSASVGDRVTITCSASSSVSYMLWFQQKPGKAPKLLIYSTSNLASGVPSRFSGSGSGTDFTLTISSLQPEDFATYYCQQRTFYPYTFGGGTKVEIK

SEQ ID NO: 57 - protein, 118 aa, Artificial Sequence
  Variable Heavy Chain
QVQLVQSGAEVKKPGASVKVSCTASGFNITDYYVHWVKQRPGQGLEWMGRIDPEDGDSKYAPKFQGKATMTADTSTSTVYMELSSLRSEDTAVYYCTTSYYVGTYGYWGQGTLVTVSS

SEQ ID NO: 58 - protein, 118 aa, Artificial Sequence
  Variable Heavy Chain in Antibody C
QVQLVQSGAEVKKPGASVKVSCTASGFNIKDYYVHWVKQAPGQGLEWMGRIDPEDGDSKYAPKFQGKATMTADTSTSTVYMELSSLRSEDTAVYYCTTSYYVGTYGYWGQGTLVTVSS

SEQ ID NO: 59 - protein, 118 aa, Artificial Sequence
  Variable Heavy Chain
QVQLVQSGAEVKKPGASVKVSCTASGFNITDYYVHWVKQRPGQGLEWMGRIDPEDGDSKYAPKFQGKVTMTADTSTSTVYMELSSLRSEDTAVYYCTTSYYVGTYGYWGQGTLVTVSS

SEQ ID NO: 60 - protein, 118 aa, Artificial Sequence
  Variable Heavy Chain
QVQLVQSGAEVKKPGASVKVSCTASGFNIKDYYVHWVKQAPGQGLEWIGRIDPEDGDSKYAPKFQGKATMTADTSTSTVYMELSSLRSEDTAVYYCTTSYYVGTYGYWGQGTLVTVSS

SEQ ID NO: 61 - protein, 118 aa, Artificial Sequence
  Variable Heavy Chain
QVQLVQSGAEVKKPGASVKVSCTASGFNITDYYVHWVKQAPGQGLEWMGRIDPEDGDSKYAPKFQGKATMTADTSTSTVYMELSSLRSEDTAVYYCTTSYYVGTYGYWGQGTLVTVSS

SEQ ID NO: 62 - protein, 118 aa, Artificial Sequence
  Variable Heavy Sequence Version 1 from Antibody 19B10-Hum
QVQLVQSGAEVKKPGASVKVSCTASGFNITDYYVHWVKQRPGQGLEWMGRIDPEDGDTKFAPKFQGKATMTADTSTSTVYMELSSLRSEDTAVYYCTTSYYVGTYGYWGQGTLVTVSS

SEQ ID NO: 63 - protein, 118 aa, Artificial Sequence
  Variable Heavy Sequence Version 2 from Antibody 19B10-Hum
QVQLVQSGAEVKKPGASVKVSCTASGFNITDYYVHWVKQRPGQGLEWMGRIDPEDGDTKFAPKFQGKVTMTADTSTSTVYMELSSLRSEDTAVYYCTTSYYVGTYGYWGQGTLVTVSS

SEQ ID NO: 64 - protein, 118 aa, Artificial Sequence
  Variable Heavy Sequence Version 3 from Antibody 19B10-Hum
QVQLVQSGAEVKKPGASVKVSCTASGFNIKDYYVHWVKQAPGQGLEWIGRIDPEDGDTKFAPKFQGKATMTADTSTSTVYMELSSLRSEDTAVYYCTTSYYVGTYGYWGQGTLVTVSS

SEQ ID NO: 65 - protein, 118 aa, Artificial Sequence
  Variable Heavy Sequence Version 4 from Antibody 19B10-Hum
QVQLVQSGAEVKKPGASVKVSCTASGFNIKDYYVHWVKQAPGQGLEWMGRIDPEDGDTKFAPKFQGKATMTADTSTSTVYMELSSLRSEDTAVYYCTTSYYVGTYGYWGQGTLVTVSS

SEQ ID NO: 66 - protein, 118 aa, Artificial Sequence
  Variable Heavy Sequence Version 5 from Antibody 19B10-Hum
QVQLVQSGAEVKKPGASVKVSCTASGFNITDYYVHWVKQAPGQGLEWMGRIDPEDGDTKFAPKFQGKATMTADTSTSTVYMELSSLRSEDTAVYYCTTSYYVGTYGYWGQGTLVTVSS

SEQ ID NO: 67 - protein, 118 aa, Artificial Sequence
  Variable Heavy Sequence Version 1 from Antibody 10F2Hum
EVQLVQSGAEVKKPGATVKISCKVSGFNIKDYYIHWVKQRPGKGLEWMGRIDPEDGDTKYDPKFQGRVTMTADTSTDTAYMELSSLRSEDTAVYYCTTSYYVGTYGYWGQGTTVTVSS

SEQ ID NO: 68 - protein, 118 aa, Artificial Sequence
  Variable Heavy Sequence Version 2 from Antibody 10F2Hum
EVQLVQSGAEVKKPGATVKISCTVSGFNIKDYYIHWVKQRPGKGLEWMGRIDPEDGDTKYDPKFQGRVTMTADTSTDTAYMELSSLRSEDTAVYYCTTSYYVGTYGYWGQGTTVTVSS

SEQ ID NO: 69 - protein, 118 aa, Artificial Sequence
  Variable Heavy Sequence Version 3 from Antibody 10F2Hum
EVQLVQSGAEVKKPGATVKISCTVSGFNIKDYYIHWVKQRPGKGLEWMGRIDPEDGDTKYDPKFQGKVTMTADTSTDTAYMELSSLRSEDTAVYYCTTSYYVGTYGYWGQGTTVTVSS

SEQ ID NO: 70 - protein, 118 aa, Artificial Sequence
  Variable Heavy Sequence Version 4 from Antibody 10F2Hum
EVQLVQSGAEVKKPGATVKISCTVSGFNIKDYYIHWVKQAPGKGLEWMGRIDPEDGDTKYDPKFQGKATMTADTSTDTAYMELSSLRSEDTAVYYCTTSYYVGTYGYWGQGTTVTVSS

SEQ ID NO: 71 - protein, 118 aa, Artificial Sequence
  Variable Heavy Sequence Version 5 from Antibody 10F2Hum
EVQLVQSGAEVKKPGATVKISCTVSGFNIKDYYIHWVKQRPGKGLEWMGRIDPEDGDTKYDPKFQGKATMTADTSTDTAYMELSSLRSEDTAVYYCTTSYYVGTYGYWGQGTTVTVSS

SEQ ID NO: 72 - protein, 118 aa, Artificial Sequence
  Variable Heavy Sequence Version 6 from Antibody 10F2Hum
EVQLVQSGAEVKKPGATVKISCTVSGFNIKDYYIHWVKQAPGKGLEWIGRIDPEDGDTKYDPKFQGKATMTADTSTDTAYMELSSLRSEDTAVYYCTTSYYVGTYGYWGQGTTVTVSS

SEQ ID NO: 73 - protein, 118 aa, Artificial Sequence
  Variable Heavy Sequence Version 7 from Antibody 10F2Hum
EVQLVQSGAEVKKPGATVKISCKVSGFNIKDYYIHWVQQAPGKGLEWMGRIDPEDGDTKYDPKFQGRVTMTADTSTDTAYMELSSLRSEDTAVYYCTTSYYVGTYGYWGQGTTVTVSS

SEQ ID NO: 74 - protein, 106 aa, Artificial Sequence
  Variable Light Sequence Version 1 from Antibody 10F2Hum
DIQMTQSPSSLSASVGDRVTITCSATSSVSYILWFQQKPGKAPKLLIYSTSNLASGVPSRFSGSGSGTDFTLTISSLQPEDFATYYCQQRTFYPYTFGGGTKVEIK

SEQ ID NO: 75 - protein, 106 aa, Artificial Sequence
  Variable Light Sequence Version 2 from Antibody 10F2Hum
DIQMTQSPSSLSASVGDRVTITCSATSSVSYILWFQQKPGKAPKLLIYSTSNLASGVPARFSGSGSGTDFTLTISSLQPEDFATYYCQQRTFYPYTFGGGTKVEIK

SEQ ID NO: 76 - protein, 106 aa, Artificial Sequence
  Variable Light Sequence Version 3 from Antibody 10F2Hum
QIQMTQSPSSLSASVGDRVTITCSATSSVSYILWFQQKPGKAPKLWIYSTSNLASGVPARFSGSGSGTDFTLTISSLQPEDFATYYCQQRTFYPYTFGGGTKVEIK

SEQ ID NO: 77 - protein, 11 aa, Artificial Sequence
  Heavy Chain CDR3 for 2H11, 10F2 and 19B10
TTSYYVGTYGY

SEQ ID NO: 78 - protein, 12 aa, Artificial Sequence
  Heavy Chain CDR3 for 20E2
ARQDGYRYAMDY